European Patent Specification EP 3 747 263 B1, published November 1, 2023. Title: New plants having a white foliage phenotype. Applicant: Klemm & Sohn GmbH & Co. KG. The sequence listing filed with the application follows.

SEQUENCE LISTING (61 sequences)

SEQ ID NO: 1 - DNA, 2314 bp, Euphorbia pulcherrima
atggtagtgaaagtgtatggagcagctcaggcagcttgcccacaaagagtaatggcctgccttttagagaaagatattccttttgatcttgttcatgttgatcttccttctgctcaacataaactctcttccttccttctcaaacaggttctttacttccctttttttactatacatttcttctaggcctaatatacatctagaccccctatagttgttcctgaaaacccctcagccccctgaacttgttaaagtggatcttacagccccttaaacttggtcaaactgaacctcaaaaccccttaatggtaacatgcccagttttgttccggtaaatcagttttcgattcaatctttgacgaaacaatcttagattcaatctttagaaaaataatacttgacatatcagcatcaagcggctatggggttcacttttaacaagttcagggtgctataaagtccactttaataaattcagggttaaggataccttttgtaagtttaggtggttgaggggttttaagggaactataggaggcctagatttattagctctcttgtttgatgtcacaattaattatgtttatttatttattctgtagccctttgggttagttccagctatagaagatggggatttcaggctttttggtatgtttcttaatcttttcatttcagtgatagccctcagtatttcgttttactaagatttcgggaccacaattcgtttttgtagtgtcactatggataattgttaaaaatgagacatgtacaaaacaaatcctattcgaatcttctatcgttggtcataaccacatggatatctacgcataaaaataccaaaaaatattttaacatgtacatgttcttttgtattccgtccactatttcgataagcatcgatttatcgttttttggctttaaattataatggactaaactaaaatgattcattaaactgtctgaacttctttattgtgaaatcacggatagctgttgcaactccacttcagggtcaattggaaacaacatctctgtaattacatgggtaaggctgcatacactcaaccccccgacactgcttgtgagggagccttattaggcattggggtgatgttgttgttttacacgttattttgtatcattgtaatctatcaaactattataattacttattaccaagtataatttattacattgattaaagtataatttattccactaaatttatgttttatgcaccttaccctgaactttgattttttatttagtattataaaatgttgtttaagtaaataaaatagatactatttaaaaataatttagaaaaaaataataaaatagagcaaggtctccatacaaaaccatcgtacttatttgaacagatatatatgtagtgttattcatatttttttttataataacatagaactgatgaatctggattagaaatgatgatataatggcttgcctcattcacgatcacacaattgataagtctgattttaccaacaaatatcagtttttcaatattatgtgttgctattttcttgaagaagaaattttgcacgaccatatttaagaataggcttagattgatcggtcaaacaaaatcttaggttattttttcattttccttttctcattagttagaatcaaaatttggaattaaattttttgttttaattttacttctaactattgagatcatatatcaccaaatatatgctttctttattatttctacataaaaaaatatatggttttacaactacctaactatgcttttttttaaagtttgcctcattaggcttacaactaccaaactatgttgaattaatataattttgtttgtgtgtgtgaagaatcaagagccataatgagatactatgcaacaaaatatgaagaaagagggcccaatttgttaggaaaaacattagaagagaaagcaatagttgatcaatgggttgaagtggaagcccataatttcaataatttggtttacaatattgtaattgaagttttgataaagccaaaaatgggggaacaaggtgacatcaacatagtcaaaagctgtgaacataagctggataaagtgttcgatgtgtacgaggaaaggctatccagttccaaatatcttggaggagattatttcacacttgctgatttaacccatatgccttccattaggtaccttgttcatgagcttgggttagcccatttggttcacaatagaaacaaggtcaatgcttggtggattgatatatcggaccgaccggcttggaaaaatttgatgattcttgctggttattag

SEQ ID NO: 2 - DNA, 645 bp, Euphorbia pulcherrima
atggtagtgaaagtgtatggagcagctcaggcagcttgcccacaaagagtaatggcctgccttttagagaaagatattccttttgatcttgttcatgttgatcttccttctgctcaacataaactctcttccttccttctcaaacagccctttgggttagttccagctatagaagatggggatttcaggctttttgaatcaagagccataatgagatactatgcaacaaaatatgaagaaagagggcccaatttgttaggaaaaacattagaagagaaagcaatagttgatcaatgggttgaagtggaagcccataatttcaataatttggtttacaatattgtaattgaagttttgataaagccaaaaatgggggaacaaggtgacatcaacatagtcaaaagctgtgaacataagctggataaagtgttcgatgtgtacgaggaaaggctatccagttccaaatatcttggaggagattatttcacacttgctgatttaacccatatgccttccattaggtaccttgttcatgagcttgggttagcccatttggttcacaatagaaacaaggtcaatgcttggtggattgatatatcggaccgaccggcttggaaaaatttgatgattcttgctggttattag

SEQ ID NO: 3 - protein, 214 aa, Euphorbia pulcherrima
MVVKVYGAAQAACPQRVMACLLEKDIPFDLVHVDLPSAQHKLSSFLLKQPFGLVPAIEDGDFRLFESRAIMRYYATKYEERGPNLLGKTLEEKAIVDQWVEVEAHNFNNLVYNIVIEVLIKPKMGEQGDINIVKSCEHKLDKVFDVYEERLSSSKYLGGDYFTLADLTHMPSIRYLVHELGLAHLVHNRNKVNAWWIDISDRPAWKNLMILAGY

SEQ ID NO: 4 - DNA, 23 bp, artificial
  amplification primer
tccgatctaagaaatcaaggcta

SEQ ID NO: 5 - DNA, 20 bp, artificial
  amplification primer
cagtcggccgctacatagat

SEQ ID NO: 6 - DNA, 20 bp, artificial
  amplification primer
tggcctgccttttagagaaa

SEQ ID NO: 7 - DNA, 20 bp, artificial
  amplification primer
aaagcctgaaatccccatct

SEQ ID NO: 8 - DNA, 20 bp, artificial
  amplification primer
tatgggcttccacttcaacc

SEQ ID NO: 9 - DNA, 37 bp, artificial
  amplification primer
gtaaaacgacggccagttggcctgccttttagagaaa

SEQ ID NO: 10 - DNA, 19 bp, artificial
  amplification primer
acaagttcagggggctgag

SEQ ID NO: 11 - DNA, 16 bp, artificial
  amplification primer
gtaaaacgacggccag

SEQ ID NO: 12 - DNA, 25 bp, artificial
  amplification primer
cctacagggaatacctcgagaatat

SEQ ID NO: 13 - DNA, 645 bp, Euphorbia pulcherrima var. Feelings Red; identical to SEQ ID NO: 2

SEQ ID NO: 14 - DNA, 645 bp, Euphorbia pulcherrima var. Glory Red
atggtagtgaaagtgtatggagcagctcaggcagcttgcccacaaagagtaatggcctgccttttagagaaagatattccttttgatctagttcatgttgatcttccttctgctcaacacaaactctcttccttccttctcaaacagccatttgggttagttccagctatagaagatggggatttcaggctttttgaatcaagagccataatgagatactatgcaacaaaatatgaagaaagagggcccaatttgttaggaaaaacattagaagagaaagcaatagttgatcaatgggttgaagtggaagcccataatttcaataatttggtttacaatattgtaattgaagttttgataaagccaaaaatgggggaacaaggtgacatcaacatagtcaaaagctgtgaacataagctggataaagtgttcgatgtgtacgaggaaaggctatccagttccaaatatcttggaggagattatttcacacttgctgatttaacccatatgccttccattaggtatcttgttcatgagcttgggttagcccatttggttcacaatagaaacaaggtcagtgcttggtggattgatatatcggacagaccggcttggaaaaatttgatgattcttgctggttattag

SEQ ID NO: 15 - DNA, 645 bp, Euphorbia pulcherrima var. Joy Red; identical to SEQ ID NO: 2

SEQ ID NO: 16 - DNA, 645 bp, Euphorbia pulcherrima var. Titan Red; identical to SEQ ID NO: 2

SEQ ID NO: 17 - DNA, 645 bp, Euphorbia pulcherrima var. Bravo Red; identical to SEQ ID NO: 14

SEQ ID NO: 18 - DNA, 645 bp, Euphorbia pulcherrima var. SK130 Red; identical to SEQ ID NO: 2

SEQ ID NO: 19 - DNA, 641 bp, Euphorbia pulcherrima var. Feelings White
atggtagtgaaagtgtatggagcagctcaggcagcttgcccacaaagagtaatggcctgccttttagagaaagatattccttttgatcttgttcatgttgatcttccttctgctcaacataaactctcttccttctcaaacagccctttgggttagttccagctatagaagatggggatttcaggctttttgaatcaagagccataatgagatactatgcaacaaaatatgaagaaagagggcccaatttgttaggaaaaacattagaagagaaagcaatagttgatcaatgggttgaagtggaagcccataatttcaataatttggtttacaatattgtaattgaagttttgataaagccaaaaatgggggaacaaggtgacatcaacatagtcaaaagctgtgaacataagctggataaagtgttcgatgtgtacgaggaaaggctatccagttccaaatatcttggaggagattatttcacacttgctgatttaacccatatgccttccattaggtaccttgttcatgagcttgggttagcccatttggttcacaatagaaacaaggtcaatgcttggtggattgatatatcggaccgaccggcttggaaaaatttgatgattcttgctggttattag

SEQ ID NO: 20 - DNA, 641 bp, Euphorbia pulcherrima var. Glory White; identical to SEQ ID NO: 19

SEQ ID NO: 21 - DNA, 641 bp, Euphorbia pulcherrima var. Joy White; identical to SEQ ID NO: 19

SEQ ID NO: 22 - DNA, 641 bp, Euphorbia pulcherrima var. Titan white; identical to SEQ ID NO: 19

SEQ ID NO: 23 - DNA, 641 bp, Euphorbia pulcherrima var. Bravo White; identical to SEQ ID NO: 19

SEQ ID NO: 24 - DNA, 641 bp, Euphorbia pulcherrima var. SK130 White; identical to SEQ ID NO: 19

SEQ ID NO: 25 - DNA, 641 bp, Euphorbia pulcherrima x Euphorbia cornastra var. Pearl; identical to SEQ ID NO: 19

SEQ ID NO: 26 - DNA, 641 bp, Euphorbia pulcherrima x Euphorbia cornastra var. Pure White; identical to SEQ ID NO: 19

SEQ ID NO: 27 - DNA, 641 bp, Euphorbia pulcherrima var. Alaska; identical to SEQ ID NO: 19

SEQ ID NO: 28 - DNA, 641 bp, Euphorbia pulcherrima var. Alpina; identical to SEQ ID NO: 19

SEQ ID NO: 29 - DNA, 585 bp, Euphorbia pulcherrima SK158 White
cagctcaggcagcttgcccacaaagagtaatggcctgccttttagagaaagatattccttttgatcttgttcatgttgatcttccttctgctcaacataaactctcttccttctcaaacagccctttgggttagttccagctatagaagatggggatttcaggctttttgaatcaagagccataatgagatactatgcaacaaaatatgaagaaagagggcccaatttgttaggaaaaacattagaagagaaagcaatagttgatcaatgggttgaagtggaagcccataatttcaataatttggtttacaatattgtaattgaagttttgataaagccaaaaatgggggaacaaggtgacatcaacatagtcaaaagctgtgaacataagctggataaagtgttcgatgtgtacgaggaaaggctatccagttccaaatatcttggaggagattatttcacacttgctgatttaacccatatgccttccattaggtaccttgttcatgagcttgggttagcccatttggttcacaatagaaacaaggtcaatgcttggtggattgatatatcggaccgaccggc

SEQ ID NO: 30 - DNA, 641 bp, Euphorbia pulcherrima Beauty White; identical to SEQ ID NO: 19

SEQ ID NO: 31 - DNA, 591 bp, Euphorbia pulcherrima x Euphorbia cornastra var. Dark Pink
ggagcagctcaggcagcttgcccacaaagagtaatggcctgccttttagagaaagatattccttttgatcttgttcatgttgatcttccttctgctcaacataaactctcttccttctcaaacagccctttgggttagttccagctatagaagatggggatttcaggctttttgaatcaagagccataatgagatactatgcaacaaaatatgaagaaagagggcccaatttgttaggaaaaacattagaagagaaagcaatagttgatcaatgggttgaagtggaagcccataatttcaataatttggtttacaatattgtaattgaagttttgataaagccaaaaatgggggaacaaggtgacatcaacatagtcaaaagctgtgaacataagctggataaagtgttcgatgtgtacgaggaaaggctatccagttccaaatatcttggaggagattatttcacacttgctgatttaacccatatgccttccattaggtaccttgttcatgagcttgggttagcccatttggttcacaatagaaacaaggtcaatgcttggtggattgatatatcggaccgaccggctg

SEQ ID NO: 32 - DNA, 641 bp, Euphorbia pulcherrima x Euphorbia cornastra var. Hot Pink; identical to SEQ ID NO: 19

SEQ ID NO: 33 - DNA, 641 bp, Euphorbia pulcherrima x Euphorbia cornastra var. Pink; identical to SEQ ID NO: 19

SEQ ID NO: 34 - DNA, 641 bp, Euphorbia pulcherrima x Euphorbia cornastra var. Soft Pink; identical to SEQ ID NO: 19

SEQ ID NO: 35 - DNA, 641 bp, Euphorbia pulcherrima var. Premium Red; identical to SEQ ID NO: 19

SEQ ID NO: 36 - DNA, 641 bp, Euphorbia pulcherrima var. Freedom Red; identical to SEQ ID NO: 19

SEQ ID NO: 37 - DNA, 641 bp, Euphorbia pulcherrima var. Otto Red; identical to SEQ ID NO: 19

SEQ ID NO: 38 - DNA, 641 bp, Euphorbia pulcherrima var. Season Red; identical to SEQ ID NO: 19

SEQ ID NO: 39 - DNA, 641 bp, Euphorbia pulcherrima var. Beauty Red; identical to SEQ ID NO: 19

SEQ ID NO: 40 - DNA, 641 bp, Euphorbia pulcherirma var. SK158 Red; identical to SEQ ID NO: 19

SEQ ID NO: 41 - DNA, 641 bp, Euphorbia pulcherrima; identical to SEQ ID NO: 19

SEQ ID NO: 42 - DNA, 645 bp, Arabidopsis thaliana
atggtggtcaaagtatatgggcagataaaagcagctaatccacaaagagtattgctctgctttttggaaaaagacatcgagtttgaagtaattcatgtcgatctcgataaacttgaacagaaaaaaccacaacatcttcttcgtcagccgtttggtcaagttccagctattgaagatggatatctgaagctttttgaatcgcgagccatagcgaggtactacgcgacaaagtatgcggaccaaggaacggacctattgggcaagactttggagggacgagccattgtggaccagtgggtggaagttgagaataactatttctacgctgtggctctacccttagttatgaacgtcgtctttaagcccaagtctggtaagccatgcgacgtcgctttggttgaggagctaaaggtcaagttcgacaaggtcctggatgtgtatgagaaccggttagctacgaaccggtacttgggcggtgatgaattcacattagctgatttgagtcatatgcccggtatgagatatatcatgaatgaaaccagtttgagtggtttggttacgtctcgagagaatctcaaccggtggtggaatgagatttcggctagaccggcttggaagaagctcatggaattggctgcctattaa

SEQ ID NO: 43 - DNA, 645 bp, Arabidopsis thaliana
atggttgtgaaactatatggacaggtaacagcagcttgtccacaaagagtcttgctttgttttctcgagaaaggaattgaatttgagattattcatatcgatcttgatacatttgagcaaaaaaaaccagaacatcttcttcgtcagccatttggtcaagttccagccatagaagatggagatttcaagctttttgaatcacgagccatcgcgagatactacgctaccaagttcgcggaccaaggcacgaaccttttgggcaagtctctagagcaccgagccatcgtggaccagtgggctgacgtggagacctattacttcaacgttctggcccaacccctcgtgattaacctaatcatcaagcctaggttaggcgagaaatgtgacgtcgttttggtcgaggatctcaaagtgaagctaggagtggtcttggacatatacaataaccggctttcttcgaaccggtttttggctggtgaagaattcactatggctgatttgacgcacatgccggcgatggggtacttgatgagtataaccgatataaaccagatggttaaggctcggggtagttttaaccggtggtgggaagagatttcggatagaccgtcttggaagaagcttatggtgctggctggtcactga

SEQ ID NO: 44 - DNA, 699 bp, Petunia x hybrida
atggttgtgaaagtgcatggttcagcaatggctgcatgcccacagagggtcatggtctgcctgatagagttgggggttgattttgagcttatccatgttgatcttgattctctcgagcagaaaaaacctgagtttctagttttacagccatttggacaagttcctgtcattgaagatggtgattttaggctttttgaatccagagcaataattaggtactatgcagcaaagtatgaagtcaagggaagcaaactaacaggaacaacattggaagagaaagctctagttgatcaatggctagaagttgaatccaataactacaatgacttagtatacaacatggtcctccaactcctagtattccccaaaatgggacaaaccagtgacttaacattggtaacaaaatgtgccaacaagttagagaatgtctttgacatttatgaacaaaggttgtcaaagagtaaatatctagcaggagagtttttctcactagctgatctaagtcaccttcctagtttaaggttcttaatgaatgaaggtggtttttcacatttggtgaccaagagaaagtgtttgcatgagtggtatttggatatttcaagtagggattcttggaagaaagtgttggacctcatgatgaagaagatatcagagattgaagcagtgtctatcccagctaaagaagaagcaaaagtttga

SEQ ID NO: 45 - DNA, 642 bp, Cyclamen persicum x Cyclamen purpurascens
atggttgttaaagtgtatggtccagccactgcaggttgcccacagagggtgatcgcttgcctttttgaacttgacgtcgactttgaaatcattcacgtcgaccttgaatccggggagcataagaagcccgattttcttcttcgccagccctttggacaagtcccagccatagaggatggagatttcaggcttttcgagtcccgggcaatcatgagatactatgcagcaaagtattccgagaagaatcctgacctacagggatcgactctagaggagaaagctctagttgaccagtggctcgaggtcgaatcacacaacttcaatgacctggtatacactctagtactccacctcatggttttccctcagatgggcaagcgcagtgacatgcagttggtacaagaatgcgagagcaaacttgagaaagtatttgatatatacgaggagagattgtcgaagagtaactacctggccggaaaattgttcacccttgccgacctcagccacctcccatctatcacttttctaatgggcgagggtgggttgggacatatggtgaggaacagaaagaacgtcaactcgtggtggatggatatttcgagcaggccttcttggaagaaggtgcggaagctgatggactag

SEQ ID NO: 46 - DNA, 642 bp, Vitis vinifera
atggtgatgaaggtgtatggcccagtgagggctgcatgcccacagagggtgttggcttgccttgtagagaagggcgtggagtttgaggttgtccatgtcgacctcgactctggcgagcaaaaacggcctgatttcctccttcgacagccttttgggcaagttccagtggtagaagatggcgatttcaggctgtttgagtcgagggcgattgtgaggtacatcgcggccaagtacgcggagcaagggcctgacctcttgggaaaaagcttggaggagaaagcggtagttgatcaatggctggaagtggaagctcacaacttcaacgagttggtgtacacactggtcatgcagctagtgatcctacctcgaatgggtgagcggggggacttggctttagcccacacttgtgagcagaagctggaaaaggtgtttgatgtgtatgagcagaggctgtcgaagagccggtaccttgcaggagattcattcactctcgctgatctgagtcatcttccggccatcagatacttggtgaaggaagctggaatggcgcacttggttactgagaggaagagtgtgagtgcatggtgggaggacatttccaacagggctgcttggaaaaaagtcatggagctcgctgcttga

SEQ ID NO: 47 - DNA, 645 bp, Litchi chinensis
atggtggttaaagtttatggaccagttacggcaggttgcccacagagagttatgacttgccttcttgaaaaagatgttgaattcgaaatcattcatgttaatatcgacaatggagagcataagcgtcctgagtttcttcttcgacagccttttgggcaagttccagtaattgaagatgacgattttaagctttttgaatcaagggcaatactgcggtactacgcggccaagtatgcggaccgtggacccaacctgcttggaaccaccctggaggagagggccagggtggaccagtggctggaagtggaagcacacaacttcaatgacttgatctacactatggtgcttcaactgatagttattccaagcatggggcagcctggggacctgacgttggtccactcctgcgagcagaagctagaggcagtttttgacgtctacgaaaagcagctttcgaagagtaagtacctcgccggagattggttctctttggcagacctcagccacatgcctgccctccggttcttgatggaggatgctaagttggtgcacctggtgaaggagaggaagcatgttaatgcgtggtgggaggagatttccggccgcctctcgtggaagaaattgatgaagcttgcctactattag

SEQ ID NO: 48 - DNA, 648 bp, Prunus persica
atggttgtgaaagtgtatggtccagtcaaggcagcctgccctcagagggttatggtttgtcttttggagaaaggagtgaatttcgaaattgttgatgttaatcttgaggtgggagagcaaaagcaacctcagttcctctcccgtcagccgtttggtcaagttccagcagtagaagatggtgatttcaggctatttgagtctagggctattatcagatactacgcagccaagtacgccgaccgtggtcccaacctattgggaacaaccctggaggagaaggctctggtggatcagtggctggaagtagaagctcacaatttcaatgacttggtttacactctggtacttcaacttctggtgctgcctcgcatgggggagcgtggtgacgtggccttggtccatgcatgtgaggagaaactggagaaggtgttcgatgtttatgaggaaagattatcaaagagcagctatctggctggagaagctttcactctggctgatctgagccatcttccagggataagctatctgattgatgaagctaaattggggcatttggtgtctgagaggaagaatgtgaatgcttggtggaaagacatatccaacaggcctgcttggaagaaactaatgagccttgctagtgactactag

SEQ ID NO: 49 - DNA, 651 bp, Prunus persica
atggttgtgaaagtgtatggtccagtcaaggcagcctgccctcagagggttatggtttgtcttttggagaaaggagtgaatttcgaaattgttgatgttaatcttgaggtgggagagcaaaagcaacctcagttcctctcccgtcagccgtttggtcaagttccagcagtagaagatggtgatttcaggctatttgagtctagggctattatcagatactacgcagccaagtacgccgaccgtggtcccaacctattgggaacaaccctggaggagaaggctctggtggatcagtggctggaagtagaagctcacaatttcaatgacttggtttacactctggtacttcaacttctggtgctgcctgatcgcatgggggagcgtggtgacgtggccttggtccatgcatgtgaggagaaactggagaaggtgttcgatgtttatgaggaaagattatcaaagagcagctatctggctggagaagctttcactctggctgatctgagccatcttccagggataagctatctgattgatgaagctaaattggggcatttggtgtctgagaggaagaatgtgaatgcttggtggaaagacatatccaacaggcctgcttggaagaaactaatgagccttgctagtgactactag

SEQ ID NO: 50 - protein, 51 aa, Euphorbia pulcherrima
MVVKVYGAAQAACPQRVMACLLEKDIPFDLVHVDLPSAQHKLSSFSNSPLG

SEQ ID NO: 51 - protein, 145 aa, Euphorbia pulcherrima
  misc_feature (145)..(145): Xaa can be any naturally occurring amino acid
MRYYATKYEERGPNLLGKTLEEKAIVDQWVEVEAHNFNNLVYNIVIEVLIKPKMGEQGDINIVKSCEHKLDKVFDVYEERLSSSKYLGGDYFTLADLTHMPSIRYLVHELGLAHLVHNRNKVNAWWIDISDRPAWKNLMILAGYX

SEQ ID NO: 52 - protein, 214 aa, Arabidopsis thaliana
MVVKVYGQIKAANPQRVLLCFLEKDIEFEVIHVDLDKLEQKKPQHLLRQPFGQVPAIEDGYLKLFESRAIARYYATKYADQGTDLLGKTLEGRAIVDQWVEVENNYFYAVALPLVMNVVFKPKSGKPCDVALVEELKVKFDKVLDVYENRLATNRYLGGDEFTLADLSHMPGMRYIMNETSLSGLVTSRENLNRWWNEISARPAWKKLMELAAY

SEQ ID NO: 53 - protein, 214 aa, Arabidopsis thaliana
MVVKLYGQVTAACPQRVLLCFLEKGIEFEIIHIDLDTFEQKKPEHLLRQPFGQVPAIEDGDFKLFESRAIARYYATKFADQGTNLLGKSLEHRAIVDQWADVETYYFNVLAQPLVINLIIKPRLGEKCDVVLVEDLKVKLGVVLDIYNNRLSSNRFLAGEEFTMADLTHMPAMGYLMSITDINQMVKARGSFNRWWEEISDRPSWKKLMVLAGH

SEQ ID NO: 54 - protein, 232 aa, Petunia x hybrida
MVVKVHGSAMAACPQRVMVCLIELGVDFELIHVDLDSLEQKKPEFLVLQPFGQVPVIEDGDFRLFESRAIIRYYAAKYEVKGSKLTGTTLEEKALVDQWLEVESNNYNDLVYNMVLQLLVFPKMGQTSDLTLVTKCANKLENVFDIYEQRLSKSKYLAGEFFSLADLSHLPSLRFLMNEGGFSHLVTKRKCLHEWYLDISSRDSWKKVLDLMMKKISEIEAVSIPAKEEAKV

SEQ ID NO: 55 - protein, 213 aa, Cyclamen persicum x Cyclamen purpurascens
MVVKVYGPATAGCPQRVIACLFELDVDFEIIHVDLESGEHKKPDFLLRQPFGQVPAIEDGDFRLFESRAIMRYYAAKYSEKNPDLQGSTLEEKALVDQWLEVESHNFNDLVYTLVLHLMVFPQMGKRSDMQLVQECESKLEKVFDIYEERLSKSNYLAGKLFTLADLSHLPSITFLMGEGGLGHMVRNRKNVNSWWMDISSRPSWKKVRKLMD

SEQ ID NO: 56 - protein, 213 aa, Vitis vinifera
MVMKVYGPVRAACPQRVLACLVEKGVEFEVVHVDLDSGEQKRPDFLLRQPFGQVPVVEDGDFRLFESRAIVRYIAAKYAEQGPDLLGKSLEEKAVVDQWLEVEAHNFNELVYTLVMQLVILPRMGERGDLALAHTCEQKLEKVFDVYEQRLSKSRYLAGDSFTLADLSHLPAIRYLVKEAGMAHLVTERKSVSAWWEDISNRAAWKKVMELAA

SEQ ID NO: 57 - protein, 214 aa, Litchi chinensis
MVVKVYGPVTAGCPQRVMTCLLEKDVEFEIIHVNIDNGEHKRPEFLLRQPFGQVPVIEDDDFKLFESRAILRYYAAKYADRGPNLLGTTLEERARVDQWLEVEAHNFNDLIYTMVLQLIVIPSMGQPGDLTLVHSCEQKLEAVFDVYEKQLSKSKYLAGDWFSLADLSHMPALRFLMEDAKLVHLVKERKHVNAWWEEISGRLSWKKLMKLAYY

SEQ ID NO: 58 - protein, 215 aa, Prunus persica
MVVKVYGPVKAACPQRVMVCLLEKGVNFEIVDVNLEVGEQKQPQFLSRQPFGQVPAVEDGDFRLFESRAIIRYYAAKYADRGPNLLGTTLEEKALVDQWLEVEAHNFNDLVYTLVLQLLVLPRMGERGDVALVHACEEKLEKVFDVYEERLSKSSYLAGEAFTLADLSHLPGISYLIDEAKLGHLVSERKNVNAWWKDISNRPAWKKLMSLASDY

SEQ ID NO: 59 - protein, 216 aa, Prunus persica
MVVKVYGPVKAACPQRVMVCLLEKGVNFEIVDVNLEVGEQKQPQFLSRQPFGQVPAVEDGDFRLFESRAIIRYYAAKYADRGPNLLGTTLEEKALVDQWLEVEAHNFNDLVYTLVLQLLVLPDRMGERGDVALVHACEEKLEKVFDVYEERLSKSSYLAGEAFTLADLSHLPGISYLIDEAKLGHLVSERKNVNAWWKDISNRPAWKKLMSLASDY

SEQ ID NO: 60 - DNA, 20 bp, artificial
  amplification primer
tggcctgccttttagagaaa

SEQ ID NO: 61 - DNA, 2351 bp, Euphorbia pulcherrima
aaaactctataacaaacaagaaatcaaggctaaaaaaatggtagtgaaagtgtatggagcagctcaggcagcttgcccacaaagagtaatggcctgccttttagagaaagatattccttttgatcttgttcatgttgatcttccttctgctcaacataaactctcttccttccttctcaaacaggttctttacttccctttttttactatacatttcttctaggcctaatatacatctagaccccctatagttgttcctgaaaacccctcagccccctgaacttgttaaagtggatcttacagccccttaaacttggtcaaactgaacctcaaaaccccttaatggtaacatgcccagttttgttccggtaaatcagttttcgattcaatctttgacgaaacaatcttagattcaatctttagaaaaataatacttgacatatcagcatcaagcggctatggggttcacttttaacaagttcagggtgctataaagtccactttaataaattcagggttaaggataccttttgtaagtttaggtggttgaggggttttaagggaactataggaggcctagatttattagctctcttgtttgatgtcacaattaattatgtttatttatttattctgtagccctttgggttagttccagctatagaagatggggatttcaggctttttggtatgtttcttaatcttttcatttcagtgatagccctcagtatttcgttttactaagatttcgggaccacaattcgtttttgtagtgtcactatggataattgttaaaaatgagacatgtacaaaacaaatcctattcgaatcttctatcgttggtcataaccacatggatatctacgcataaaaataccaaaaaatattttaacatgtacatgttcttttgtattccgtccactatttcgataagcatcgatttatcgttttttggctttaaattataatggactaaactaaaatgattcattaaactgtctgaacttctttattgtgaaatcacggatagctgttgcaactccacttcagggtcaattggaaacaacatctctgtaattacatgggtaaggctgcatacactcaaccccccgacactgcttgtgagggagccttattaggcattggggtgatgttgttgttttacacgttattttgtatcattgtaatctatcaaactattataattacttattaccaagtataatttattacattgattaaagtataatttattccactaaatttatgttttatgcaccttaccctgaactttgattttttatttagtattataaaatgttgtttaagtaaataaaatagatactatttaaaaataatttagaaaaaaataataaaatagagcaaggtctccatacaaaaccatcgtacttatttgaacagatatatatgtagtgttattcatatttttttttataataacatagaactgatgaatctggattagaaatgatgatataatggcttgcctcattcacgatcacacaattgataagtctgattttaccaacaaatatcagtttttcaatattatgtgttgctattttcttgaagaagaaattttgcacgaccatatttaagaataggcttagattgatcggtcaaacaaaatcttaggttattttttcattttccttttctcattagttagaatcaaaatttggaattaaattttttgttttaattttacttctaactattgagatcatatatcaccaaatatatgctttctttattatttctacataaaaaaatatatggttttacaactacctaactatgcttttttttaaagtttgcctcattaggcttacaactaccaaactatgttgaattaatataattttgtttgtgtgtgtgaagaatcaagagccataatgagatactatgcaacaaaatatgaagaaagagggcccaatttgttaggaaaaacattagaagagaaagcaatagttgatcaatgggttgaagtggaagcccataatttcaataatttggtttacaatattgtaattgaagttttgataaagccaaaaatgggggaacaaggtgacatcaacatagtcaaaagctgtgaacataagctggataaagtgttcgatgtgtacgaggaaaggctatccagttccaaatatcttggaggagattatttcacacttgctgatttaacccatatgccttccattaggtaccttgttcatgagcttgggttagcccatttggttcacaatagaaacaaggtcaatgcttggtggattgatatatcggaccgaccggcttggaaaaatttgatgattcttgctggttattag